European Patent Application EP 4 389 899 A1, published June 26, 2024. Title: Regulatory Nucleic Acid Sequences. Applicant: Synpromics Limited. Application GR. The sequence listing filed with the application follows.

SEQUENCE LISTING (26 sequences)

SEQ ID NO: 1 - DNA, 348 bp, synthetic construct
  source 1..348: mol_type = other DNA
  misc_feature 1..348: note = SP0525
gctgcccatgtaaggaggcaaggcctggggacacccgagatgcctggttataattaacccagacatgtggctgccccccccccccaacacctgctgcctctaaaaataaccctgttctcctctataaatacccgctctggtatttggggttggcagctgttgaggatacaagtgacccctgctctgttaattattggcaaattgcctaacttcaacgtaaggaaatagagtcatatgtttgctcactgaaggttactagttgtacttatataagggggtgggggcgcgttcgtcctcagtcgcgatcgaacactcgagccgagcagacgtgcctacggaccggccacc

SEQ ID NO: 2 - DNA, 302 bp, synthetic construct
  source 1..302: mol_type = other DNA
  misc_feature 1..302: note = SP0526
gctgcccatgtaaggaggcaaggcctggggacacccgagatgcctggttataattaacccagacatgtggctgccccccccccccaacacctgctgcctctaaaaataaccctgttctcctctataaatacccgctctggtatttggggttggcagctgttgttggcaaattgcctaacttcaacgtaaggaaatagagtcatatgtttgctcacgtacttatataagggggtgggggcgcgttcgtcctcagtcgcgatcgaacactcgagccgagcagacgtgcctacggaccggccacc

SEQ ID NO: 3 - DNA, 280 bp, synthetic construct
  source 1..280: mol_type = other DNA
  misc_feature 1..280: note = SP0527
gctgcccatgtaaggaggcaaggcctggggacacccgagatgcctggttataattaacccagacatgtggctgccccccccccccaacacctgctgcctctaaaaataaccctgttctcctctataaatacccgctctggtatttggggttggcagctgttggcctaacttcaacgtaaggaaatagagtcatgtacttatataagggggtgggggcgcgttcgtcctcagtcgcgatcgaacactcgagccgagcagacgtgcctacggaccggccacc

SEQ ID NO: 4 - DNA, 311 bp, synthetic construct
  source 1..311: mol_type = other DNA
  misc_feature 1..311: note = SP0528
gctgcccatgtaaggaggcaaggcctggggacacccgagatgcctggttataattaacccagacatgtggctgccccccccccccaacacctgctgcctctaaaaataaccctggcctaacttcaacgtaaggaaatagagtcatttctcctctataaatacccgctctggtatttggggttggcagctgttggcctaacttcaacgtaaggaaatagagtcatgtacttatataagggggtgggggcgcgttcgtcctcagtcgcgatcgaacactcgagccgagcagacgtgcctacggaccggccacc

SEQ ID NO: 5 - DNA, 19 bp, synthetic construct
  source 1..19: mol_type = other DNA
  misc_feature 1..19: note = mGapdH FW Primer
acggcaaattcaacggcac

SEQ ID NO: 6 - DNA, 24 bp, synthetic construct
  source 1..24: mol_type = other DNA
  misc_feature 1..24: note = mGapdH Probe
  misc_feature 1: note = JOE 5' reporter dye
  misc_feature 24: note = BHQ1 3' quencher
ttgtcatcaacgggaagcccatca

SEQ ID NO: 7 - DNA, 249 bp, synthetic construct
  source 1..249: mol_type = other DNA
  misc_feature 1..249: note = SP0524
gctgcccatgtaaggaggcaaggcctggggacacccgagatgcctggttataattaacccagacatgtggctgccccccccccccaacacctgctgcctctaaaaataaccctgttctcctctataaatacccgctctggtatttggggttggcagctgttggtacttatataagggggtgggggcgcgttcgtcctcagtcgcgatcgaacactcgagccgagcagacgtgcctacggaccggccacc

SEQ ID NO: 8 - DNA, 162 bp, synthetic construct
  source 1..162: mol_type = other DNA
  misc_feature 1..162: note = CRM from SP0524, SP0530 and SP0531
gctgcccatgtaaggaggcaaggcctggggacacccgagatgcctggttataattaacccagacatgtggctgccccccccccccaacacctgctgcctctaaaaataaccctgttctcctctataaatacccgctctggtatttggggttggcagctgttg

SEQ ID NO: 9 - DNA, 224 bp, synthetic construct
  source 1..224: mol_type = other DNA
  misc_feature 1..224: note = CRM_ SP0528
gctgcccatgtaaggaggcaaggcctggggacacccgagatgcctggttataattaacccagacatgtggctgccccccccccccaacacctgctgcctctaaaaataaccctggcctaacttcaacgtaaggaaatagagtcatttctcctctataaatacccgctctggtatttggggttggcagctgttggcctaacttcaacgtaaggaaatagagtcat

SEQ ID NO: 10 - DNA, 114 bp, synthetic construct
  source 1..114: mol_type = other DNA
  misc_feature 1..114: note = CRE0145
gctgcccatgtaaggaggcaaggcctggggacacccgagatgcctggttataattaacccagacatgtggctgccccccccccccaacacctgctgcctctaaaaataaccctg

SEQ ID NO: 11 - DNA, 48 bp, synthetic construct
  source 1..48: mol_type = other DNA
  misc_feature 1..48: note = DES_MT_enhancer_48bp
ttctcctctataaatacccgctctggtatttggggttggcagctgttg

SEQ ID NO: 12 - DNA, 81 bp, synthetic construct
  source 1..81: mol_type = other DNA
  misc_feature 1..81: note = SCP1
gtacttatataagggggtgggggcgcgttcgtcctcagtcgcgatcgaacactcgagccgagcagacgtgcctacggaccg

SEQ ID NO: 13 - DNA, 99 bp, synthetic construct
  source 1..99: mol_type = other DNA
  misc_feature 1..99: note = Liver de-targeting sequence 1
aggatacaagtgacccctgctctgttaattattggcaaattgcctaacttcaacgtaaggaaatagagtcatatgtttgctcactgaaggttactagtt

SEQ ID NO: 14 - DNA, 53 bp, synthetic construct
  source 1..53: mol_type = other DNA
  misc_feature 1..53: note = Liver de-targeting sequence 2
ttggcaaattgcctaacttcaacgtaaggaaatagagtcatatgtttgctcac

SEQ ID NO: 15 - DNA, 19 bp, synthetic construct
  source 1..19: mol_type = other DNA
  misc_feature 1..19: note = ZBTB20 binding site
cttcaacgtaaggaaatag

SEQ ID NO: 16 - DNA, 76 bp, synthetic construct
  source 1..76: mol_type = other DNA
  misc_feature 1..76: note = Mir122 miRNA target sequence 1
caaacaccattgtcacactccatcaccaaacaccattgtcacactccagatatccaaacaccattgtcacactcca

SEQ ID NO: 17 - DNA, 31 bp, synthetic construct
  source 1..31: mol_type = other DNA
  misc_feature 1..31: note = Liver de-targeting sequence 3
gcctaacttcaacgtaaggaaatagagtcat

SEQ ID NO: 18 - DNA, 20 bp, synthetic construct
  source 1..20: mol_type = other DNA
  misc_feature 1..20: note = mGapdH Primer RV
tagtggggtctcgctcctgg

SEQ ID NO: 19 - DNA, 22 bp, synthetic construct
  source 1..22: mol_type = other DNA
  misc_feature 1..22: note = Mir122 miRNA target sequence 2
caaacaccattgtcacactcca

SEQ ID NO: 20 - DNA, 261 bp, synthetic construct
  source 1..261: mol_type = other DNA
  misc_feature 1..261: note = CRM_SP0525
gctgcccatgtaaggaggcaaggcctggggacacccgagatgcctggttataattaacccagacatgtggctgccccccccccccaacacctgctgcctctaaaaataaccctgttctcctctataaatacccgctctggtatttggggttggcagctgttgaggatacaagtgacccctgctctgttaattattggcaaattgcctaacttcaacgtaaggaaatagagtcatatgtttgctcactgaaggttactagtt

SEQ ID NO: 21 - DNA, 215 bp, synthetic construct
  source 1..215: mol_type = other DNA
  misc_feature 1..215: note = CRM_SP0526
gctgcccatgtaaggaggcaaggcctggggacacccgagatgcctggttataattaacccagacatgtggctgccccccccccccaacacctgctgcctctaaaaataaccctgttctcctctataaatacccgctctggtatttggggttggcagctgttgttggcaaattgcctaacttcaacgtaaggaaatagagtcatatgtttgctcac

SEQ ID NO: 22 - DNA, 193 bp, synthetic construct
  source 1..193: mol_type = other DNA
  misc_feature 1..193: note = CRM_ SP0527
gctgcccatgtaaggaggcaaggcctggggacacccgagatgcctggttataattaacccagacatgtggctgccccccccccccaacacctgctgcctctaaaaataaccctgttctcctctataaatacccgctctggtatttggggttggcagctgttggcctaacttcaacgtaaggaaatagagtcat

SEQ ID NO: 23 - DNA, 18 bp, synthetic construct
  source 1..18: mol_type = other DNA
  misc_feature 1..18: note = Luc2 Fw Primer
acgctgggctacttgatc

SEQ ID NO: 24 - DNA, 18 bp, synthetic construct
  source 1..18: mol_type = other DNA
  misc_feature 1..18: note = Luc2 Probe
  misc_feature 1: note = FAM 5' reporter dye
  misc_feature 18: note = BHQ1 3'quencher
tttcgggtcgtgctcatg

SEQ ID NO: 25 - DNA, 19 bp, synthetic construct
  source 1..19: mol_type = other DNA
  misc_feature 1..19: note = Luc2 RV Primer
caagaatagctcctcctcg

SEQ ID NO: 26 - DNA, 69 bp, synthetic construct
  source 1..69: mol_type = other DNA
  misc_feature 1..69: note = CRE0053
caccgcctgctgccacggccggccgtataaatagaggcgaggagcagctgggctctcttggcagtcacc